European Patent Application EP 4 786 592 A1, published August 5, 2026. Title: Nucleic acid molecule comprising modified polyadenyl sequence and OX40L protein coding sequence. Applicant: HANMI PHARM. CO., LTD. The sequence listing filed with the application follows.

SEQUENCE LISTING (27 sequences)

SEQ ID NO: 1 - DNA, 158 bp, Homo sapiens
  source 1..158: mol_type = genomic DNA
gtgtgtggaggacaccctgaaccccccgctttcaaacaagttttcaaattgtttgaggtcaggatttctcaaactgattcctttctttgcatatgagtatttgaaaataaatattttcccagaatataaataaatcatcacatgattattttaactat

SEQ ID NO: 2 - DNA, 142 bp, synthetic construct
  source 1..142: mol_type = other DNA
aaaaaaaaaaaaaaaaaaaaacaaccagctaagacactgccaaaaaaaaaaaaaaaaaaaaaaaaaaaaaaaaaaaaaaaaaaaaaaaaaaaaaaaaaaaaaaaaaaaaaaaaaaaaaaaaaaaaaaaaaaaaaaaaaaaaa

SEQ ID NO: 3 - DNA, 3103 bp, synthetic construct
  source 1..3103: mol_type = other DNA
aagcttctcgaggtgtgtggaggacaccctgaaccccccgctttcaaacaagttttcaaattgtttgaggtcaggatttctcaaactgattcctttctttgcatatgagtatttgaaaataaatattttcccagaatataaataaatcatcacatgattattttaactatgctagcaaaaaaaaaaaaaaaaaaaaacaaccagctaagacactgccaaaaaaaaaaaaaaaaaaaaaaaaaaaaaaaaaaaaaaaaaaaaaaaaaaaaaaaaaaaaaaaaaaaaaaaaaaaaaaaaaaaaaaaaaaaaaaaaaaaaagaagagcgaattcactggccgtcgttttacagttacccaacttaatcgcctcgcctgatgcggtattttctccttacgcatctgtgcggtatttcacaccgcatatggtgcactctcagtacaatctgctctgatgccgcatagttaagccagccccgacacccgccaacacccgctgacgcgccctgacgggcttgtctgctcccggcatccgcttacagacaagctgtgaccgtctccgggagctgcatgtgtcagaggttttcaccgtcatcaccgaaacgcgcgagacgaaagggcctcgtgatacgcctatttttataggttaatgtcatgataataatggtttcttagacgtcaggtggcacttttcggggaaatgtgcgcggaacccctatttgtttatttttctaaatacattcaaatatgtatccgctcatgagacaataaccctgataaatgcttcaataatattgaaaaagtatgagtattcaacatttccgtgtcgcccttattcccttttttgcggcattttgccttcctgtttttgctcacccagaaacgctggtgaaagtaaaagatgctgaagatcagttgggtgcacgagtgggttacatcgaactggatctcaacagcggtaagatccttgagagttttcgccccgaagaacgttttccatgcagctctggcccgtgtctcaaaatctctgatgttacattgcacaagataaaaatatatcatcatgaacaataaaactgtctgcttacataaacagtaatacaaggggtgttatgagccatattcaacgggaaacgtcgaggccgcgattaaattccaacatggatgctgatttatatgggtataaatgggctcgcgataatgtcgggcaatcaggtgcgacaatctatcgcttgtatgggaagcccgatgcgccagagttgtttctgaaacatggcaaaggtagcgttgccaatgatgttacagatgagatggtcagactaaactggctgacggaatttatgcctcttccgaccatcaagcattttatccgtactcctgatgatgcatggttactcaccactgcgatccccggaaaaacagcattccaggtattagaagaatatcctgattcaggtgaaaatattgttgatgcgctggcagtgttcctgcgccggttgcattcgattcctgtttgtaattgtccttttaacagcgatcgcgtatttcgtctcgctcaggcgcaatcacgaatgaataacggtttggttgatgcgagtgattttgatgacgagcgtaatggctggcctgttgaacaagtctggaaagaaatgcataaacttttgccattctcaccggattcagtcgtcactcatggtgatttctcacttgataaccttatttttgacgaggggaaattaataggttgtattgatgttggacgagtcggaatcgcagaccgataccaggatcttgccatcctatggaactgcctcggtgagttttctccttcattacagaaacggctttttcaaaaatatggtattgataatcctgatatgaataaattgcagtttcatttgatgctcgatgagtttttctaatcagaattggttaattggttgtaacattattcagattgggcttgatttaaaacttcatttttaatttaaaaggatctaggtgaagatcctttttgataatctcatgaccaaaatcccttaacgtgagttttcgttccactgagcgtcagaccccgtagaaaagatcaaaggatcttcttgagatcctttttttctgcgcgtaatctgctgcttgcaaacaaaaaaaccaccgctaccagcggtggtttgtttgccggatcaagagctaccaactctttttccgaaggtaactggcttcagcagagcgcagataccaaatactgttcttctagtgtagccgtagttaggccaccacttcaagaactctgtagcaccgcctacatacctcgctctgctaatcctgttaccagtggctgctgccagtggcgataagtcgtgtcttaccgggttggactcaagacgatagttaccggataaggcgcagcggtcgggctgaacggggggttcgtgcacacagcccagcttggagcgaacgacctacaccgaactgagatacctacagcgtgagctatgagaaagcgccacgcttcccgaagggagaaaggcggacaggtatccggtaagcggcagggtcggaacaggagagcgcacgagggagcttccagggggaaacgcctggtatctttatagtcctgtcgggtttcgccacctctgacttgagcgtcgatttttgtgatgctcgtcaggggggcggagcctatggaaaaacgccagcaacgcggcctttttacggttcctggccttttgctggccttttgcgagccttttgctcacatgttctttcctgcgttatcccctgattctgtggataaccgtattaccgcctttgagtgagctgataccgctcgccgcagccgaacgaccgagcgcagcgagtcagtgagcgaggaagcggcccaatacgcaaaccgcctctccccgcgcgttggccgattcattaatgcagctggcacgacaggtttcccgactggaaagcgggcagtgagcgcaacgcaattaatgtgagttagctcactcattaggcaccccaggctttacactttatgcttccggctcgtatgttgtgtggaattgtgagcggataacaatttcacacaggaaacagctatgaccatgattacgcc

SEQ ID NO: 4 - DNA, 3079 bp, synthetic construct
  source 1..3079: mol_type = other DNA
gtgtgtggaggacaccctgaaccccccgctttcaaacaagttttcaaattgtttgaggtcaggatttctcaaactgattcctttctttgcatatgagtatttgaaaataaatattttcccagaatataaataaatcatcacatgattattttaactataaaaaaaaaaaaaaaaaaaaacaaccagctaagacactgccaaaaaaaaaaaaaaaaaaaaaaaaaaaaaaaaaaaaaaaaaaaaaaaaaaaaaaaaaaaaaaaaaaaaaaaaaaaaaaaaaaaaaaaaaaaaaaaaaaaaagaagagcactggccgtcgttttacagttacccaacttaatcgcctcgcctgatgcggtattttctccttacgcatctgtgcggtatttcacaccgcatatggtgcactctcagtacaatctgctctgatgccgcatagttaagccagccccgacacccgccaacacccgctgacgcgccctgacgggcttgtctgctcccggcatccgcttacagacaagctgtgaccgtctccgggagctgcatgtgtcagaggttttcaccgtcatcaccgaaacgcgcgagacgaaagggcctcgtgatacgcctatttttataggttaatgtcatgataataatggtttcttagacgtcaggtggcacttttcggggaaatgtgcgcggaacccctatttgtttatttttctaaatacattcaaatatgtatccgctcatgagacaataaccctgataaatgcttcaataatattgaaaaagtatgagtattcaacatttccgtgtcgcccttattcccttttttgcggcattttgccttcctgtttttgctcacccagaaacgctggtgaaagtaaaagatgctgaagatcagttgggtgcacgagtgggttacatcgaactggatctcaacagcggtaagatccttgagagttttcgccccgaagaacgttttccatgcagctctggcccgtgtctcaaaatctctgatgttacattgcacaagataaaaatatatcatcatgaacaataaaactgtctgcttacataaacagtaatacaaggggtgttatgagccatattcaacgggaaacgtcgaggccgcgattaaattccaacatggatgctgatttatatgggtataaatgggctcgcgataatgtcgggcaatcaggtgcgacaatctatcgcttgtatgggaagcccgatgcgccagagttgtttctgaaacatggcaaaggtagcgttgccaatgatgttacagatgagatggtcagactaaactggctgacggaatttatgcctcttccgaccatcaagcattttatccgtactcctgatgatgcatggttactcaccactgcgatccccggaaaaacagcattccaggtattagaagaatatcctgattcaggtgaaaatattgttgatgcgctggcagtgttcctgcgccggttgcattcgattcctgtttgtaattgtccttttaacagcgatcgcgtatttcgtctcgctcaggcgcaatcacgaatgaataacggtttggttgatgcgagtgattttgatgacgagcgtaatggctggcctgttgaacaagtctggaaagaaatgcataaacttttgccattctcaccggattcagtcgtcactcatggtgatttctcacttgataaccttatttttgacgaggggaaattaataggttgtattgatgttggacgagtcggaatcgcagaccgataccaggatcttgccatcctatggaactgcctcggtgagttttctccttcattacagaaacggctttttcaaaaatatggtattgataatcctgatatgaataaattgcagtttcatttgatgctcgatgagtttttctaatcagaattggttaattggttgtaacattattcagattgggcttgatttaaaacttcatttttaatttaaaaggatctaggtgaagatcctttttgataatctcatgaccaaaatcccttaacgtgagttttcgttccactgagcgtcagaccccgtagaaaagatcaaaggatcttcttgagatcctttttttctgcgcgtaatctgctgcttgcaaacaaaaaaaccaccgctaccagcggtggtttgtttgccggatcaagagctaccaactctttttccgaaggtaactggcttcagcagagcgcagataccaaatactgttcttctagtgtagccgtagttaggccaccacttcaagaactctgtagcaccgcctacatacctcgctctgctaatcctgttaccagtggctgctgccagtggcgataagtcgtgtcttaccgggttggactcaagacgatagttaccggataaggcgcagcggtcgggctgaacggggggttcgtgcacacagcccagcttggagcgaacgacctacaccgaactgagatacctacagcgtgagctatgagaaagcgccacgcttcccgaagggagaaaggcggacaggtatccggtaagcggcagggtcggaacaggagagcgcacgagggagcttccagggggaaacgcctggtatctttatagtcctgtcgggtttcgccacctctgacttgagcgtcgatttttgtgatgctcgtcaggggggcggagcctatggaaaaacgccagcaacgcggcctttttacggttcctggccttttgctggccttttgcgagccttttgctcacatgttctttcctgcgttatcccctgattctgtggataaccgtattaccgcctttgagtgagctgataccgctcgccgcagccgaacgaccgagcgcagcgagtcagtgagcgaggaagcggcccaatacgcaaaccgcctctccccgcgcgttggccgattcattaatgcagctggcacgacaggtttcccgactggaaagcgggcagtgagcgcaacgcaattaatgtgagttagctcactcattaggcaccccaggctttacactttatgcttccggctcgtatgttgtgtggaattgtgagcggataacaatttcacacaggaaacagctatgaccatgattacgcc

SEQ ID NO: 5 - DNA, 17 bp, synthetic construct
  source 1..17: mol_type = other DNA
taatacgactcactata

SEQ ID NO: 6 - DNA, 61 bp, synthetic construct
  source 1..61: mol_type = other DNA
agtgctccccatccaactaaactgtccctctgtccgaactaaactgcactgtcccagcacc

SEQ ID NO: 7 - RNA, 61 nt, synthetic construct
  source 1..61: mol_type = other RNA
agtgctccccatccaactaaactgtccctctgtccgaactaaactgcactgtcccagcacc

SEQ ID NO: 8 - RNA, 155 nt, synthetic construct
  source 1..155: mol_type = other RNA
aaaaaaaaaaaaaaaaaaaaacaaccagctaagacactgccaaaaaaaaaaaaaaaaaaaaaaaaaaaaaaaaaaaaaaaaaaaaaaaaaaaaaaaaaaaaaaaaaaaaaaaaaaaaaaaaaaaaaaaaaaaaaaaaaaaaaagaagagcgaatt

SEQ ID NO: 9 - RNA, 158 nt, Homo sapiens
  source 1..158: mol_type = mRNA
gtgtgtggaggacaccctgaaccccccgctttcaaacaagttttcaaattgtttgaggtcaggatttctcaaactgattcctttctttgcatatgagtatttgaaaataaatattttcccagaatataaataaatcatcacatgattattttaactat

SEQ ID NO: 10 - RNA, 142 nt, synthetic construct
  source 1..142: mol_type = other RNA
aaaaaaaaaaaaaaaaaaaaacaaccagctaagacactgccaaaaaaaaaaaaaaaaaaaaaaaaaaaaaaaaaaaaaaaaaaaaaaaaaaaaaaaaaaaaaaaaaaaaaaaaaaaaaaaaaaaaaaaaaaaaaaaaaaaaa

SEQ ID NO: 11 - DNA, 57 bp, Homo sapiens
  source 1..57: mol_type = genomic DNA
atgacaaggttgacggtcctggcattgcttgccgggcttttggcgagttctcgggcg

SEQ ID NO: 12 - DNA, 444 bp, Homo sapiens
  source 1..444: mol_type = genomic DNA
agcagttcacctgcaaaggaccccccaatccagcgactgagaggcgcagtcacccggtgtgaagatggacagctttttatatcatcttacaagaatgagtatcagactatggaggttcaaaataactccgtggttataaagtgcgacgggctttacatcatctatctgaaggggtcctttttccaggaggtcaagatagatttgcacttcagggaagaccataaccccatttctattcctatgcttaatgacggacgacggatcgtatttactgttgtggcttctctcgcttttaaggacaaggtctaccttaccgtgaatgccccagacacactttgcgagcacctccagatcaacgacggagagcttatcgttgttcaacttacaccaggttattgcgctccagaggggagctatcactccaccgtcaaccaggtacccctt

SEQ ID NO: 13 - DNA, 30 bp, synthetic construct
  source 1..30: mol_type = other DNA
ggtggaggcggttcaggcggaggtggctct

SEQ ID NO: 14 - DNA, 60 bp, synthetic construct
  source 1..60: mol_type = other DNA
agcgagagaaaggcccttcagacagaaatggcacgcataaaaaaatggcttacattcagt

SEQ ID NO: 15 - DNA, 441 bp, Homo sapiens
  source 1..441: mol_type = genomic DNA
caggactccgaagcagcaataaaccgacaaataaatctggagttgtacgcatcctacgtttacctgtccatgtcttactacttcgatagagacgatgtcgccctcaaaaacttcgccaagtatttcctgcatcagtcccatgaagagagagagcacgcagagaaactgatgaaacttcagaaccaacgggggggcaggatctttctgcaagacattaagaagcctgattgcgatgactgggaatctggacttaatgccatggagtgtgccctgcacctcgaaaaaaatgtgaaccagagcctgttggaattgcataagctggcaaccgataagaacgatccacatctttgcgatttcatcgaaacccactatctcaatgaacaagtgaaggcaattaaggagctgggcgatcatgtaacaaatttgcgaaaaatgggtgcc

SEQ ID NO: 16 - DNA, 312 bp, Homo sapiens
  source 1..312: mol_type = genomic DNA
tctggctctcagacttgtgaagatacccttaagacttgcagtgtcatagcctgtgggcgagacgggcgcgatggacccaagggcgaaaaaggagaaccagggcaagggctcagaggactgcaaggtccacctggtaaattggggccacctggaagcgtggggtccccaggaagtccaggcccaaaaggtcagaaaggggaccacggcgataatcgagccattgaggaaaaactcgcaaatatggaggccgaaattaggattctgaagagtaagttgcagctgaccaacaagctccatgcttttagcatgggc

SEQ ID NO: 17 - RNA, 57 nt, Homo sapiens
  source 1..57: mol_type = mRNA
atgacaaggttgacggtcctggcattgcttgccgggcttttggcgagttctcgggcg

SEQ ID NO: 18 - RNA, 444 nt, Homo sapiens
  source 1..444: mol_type = mRNA
agcagttcacctgcaaaggaccccccaatccagcgactgagaggcgcagtcacccggtgtgaagatggacagctttttatatcatcttacaagaatgagtatcagactatggaggttcaaaataactccgtggttataaagtgcgacgggctttacatcatctatctgaaggggtcctttttccaggaggtcaagatagatttgcacttcagggaagaccataaccccatttctattcctatgcttaatgacggacgacggatcgtatttactgttgtggcttctctcgcttttaaggacaaggtctaccttaccgtgaatgccccagacacactttgcgagcacctccagatcaacgacggagagcttatcgttgttcaacttacaccaggttattgcgctccagaggggagctatcactccaccgtcaaccaggtacccctt

SEQ ID NO: 19 - RNA, 30 nt, synthetic construct
  source 1..30: mol_type = other RNA
ggtggaggcggttcaggcggaggtggctct

SEQ ID NO: 20 - RNA, 60 nt, synthetic construct
  source 1..60: mol_type = other RNA
agcgagagaaaggcccttcagacagaaatggcacgcataaaaaaatggcttacattcagt

SEQ ID NO: 21 - RNA, 441 nt, Homo sapiens
  source 1..441: mol_type = mRNA
caggactccgaagcagcaataaaccgacaaataaatctggagttgtacgcatcctacgtttacctgtccatgtcttactacttcgatagagacgatgtcgccctcaaaaacttcgccaagtatttcctgcatcagtcccatgaagagagagagcacgcagagaaactgatgaaacttcagaaccaacgggggggcaggatctttctgcaagacattaagaagcctgattgcgatgactgggaatctggacttaatgccatggagtgtgccctgcacctcgaaaaaaatgtgaaccagagcctgttggaattgcataagctggcaaccgataagaacgatccacatctttgcgatttcatcgaaacccactatctcaatgaacaagtgaaggcaattaaggagctgggcgatcatgtaacaaatttgcgaaaaatgggtgcc

SEQ ID NO: 22 - RNA, 170 nt, synthetic construct
  source 1..170: mol_type = other RNA
ctcgaggtgtgtggaggacaccctgaaccccccgctttcaaacaagttttcaaattgtttgaggtcaggatttctcaaactgattcctttctttgcatatgagtatttgaaaataaatattttcccagaatataaataaatcatcacatgattattttaactatgctagc

SEQ ID NO: 23 - RNA, 312 nt, Homo sapiens
  source 1..312: mol_type = other RNA
tctggctctcagacttgtgaagatacccttaagacttgcagtgtcatagcctgtgggcgagacgggcgcgatggacccaagggcgaaaaaggagaaccagggcaagggctcagaggactgcaaggtccacctggtaaattggggccacctggaagcgtggggtccccaggaagtccaggcccaaaaggtcagaaaggggaccacggcgataatcgagccattgaggaaaaactcgcaaatatggaggccgaaattaggattctgaagagtaagttgcagctgaccaacaagctccatgcttttagcatgggc

SEQ ID NO: 24 - protein, 349 aa, synthetic construct
MTRLTVLALLAGLLASSRASSSPAKDPPIQRLRGAVTRCEDGQLFISSYKNEYQTMEVQNNSVVIKCDGLYIIYLKGSFFQEVKIDLHFREDHNPISIPMLNDGRRIVFTVVASLAFKDKVYLTVNAPDTLCEHLQINDGELIVVQLTPGYCAPEGSYHSTVNQVPLGGGGSGGGGSSERKALQTEMARIKKWLTFSGGGGSQDSEAAINRQINLELYASYVYLSMSYYFDRDDVALKNFAKYFLHQSHEEREHAEKLMKLQNQRGGRIFLQDIKKPDCDDWESGLNAMECALHLEKNVNQSLLELHKLATDKNDPHLCDFIETHYLNEQVKAIKELGDHVTNLRKMGA

SEQ ID NO: 25 - protein, 281 aa, synthetic construct
MTRLTVLALLAGLLASSRASGSQTCEDTLKTCSVIACGRDGRDGPKGEKGEPGQGLRGLQGPPGKLGPPGSVGSPGSPGPKGQKGDHGDNRAIEEKLANMEAEIRILKSKLQLTNKLHAFSMGGGGGSGGGGSSSSPAKDPPIQRLRGAVTRCEDGQLFISSYKNEYQTMEVQNNSVVIKCDGLYIIYLKGSFFQEVKIDLHFREDHNPISIPMLNDGRRIVFTVVASLAFKDKVYLTVNAPDTLCEHLQINDGELIVVQLTPGYCAPEGSYHSTVNQVPL

SEQ ID NO: 26 - DNA, 15 bp, synthetic construct
  source 1..15: mol_type = other DNA
ggtggaggcggttca

SEQ ID NO: 27 - RNA, 15 nt, synthetic construct
  source 1..15: mol_type = other RNA
ggtggaggcggttca